European Patent Specification EP 4 025 253 B1, published March 20, 2024. Title: Drug Antibody Conjugates. Applicant: Pharma Mar, S.A. The sequence listing filed with the application follows.

SEQUENCE LISTING (3 sequences)

SEQ ID NO: 1 - protein, 5 aa, Homo sapiens
ARHCL

SEQ ID NO: 2 - protein, 4 aa, Homo sapiens
QNGS

SEQ ID NO: 3 - protein, 11 aa, Homo sapiens
PPFCVARCPSG